European Patent Application EP 4 450 647 A2, published October 23, 2024. Title: EARLY RISKASSESSMENT OFPRETERM DELIVERY INA SUBJECT. Applicant: TATA CONSULTANCY SERVICES LTD. Application EP. The sequence listing filed with the application follows.

SEQUENCE LISTING (24 sequences)

SEQ ID NO: 1 - RNA, 1442 nt, unidentified
  source 1..1442: mol_type = rRNA
gagtttgatcctggctcagggtgaacgctagcggtgcgcctaacacatgcaagtcgagcggaattgatatgttgaaagcttcggtgggaaatatattgagagagcggcgaacgggtgaggaacacgttggaatctgcccccaagtcagggatagcccagggaaacctggattaataccggatagtctctttggagtaaagatttattgcttggggaggagcctgcgtactatcagctagttggtagggtaaaagcctaccaaggcaatgacggataactggtctgagaggatgatcagtcacaatggaactgagacacggtccatactcctacgggaggcagcagtgaggaatcttccacaatgggcgaaagcctgatggagcgacaccgcgtgaaggaagaaggcctaacggttgtaaacttcttttctgaaggagcataatgagagtactttaggaataagggacggctaaatacgtgccagcagccgcggtaatacgtatgtctcgagcgttacccggaattactgggtgtaaagggtttgtaggttggtgaataagtcaggtatgaaagaccggagcttaactccgagtttgtgcttgaaactgttgacctagaatcagggagaggtaagcggaattctaagtgtaggggtgcaatccgtagatacttagaggaacaccaaaagcgaaggcagcttactggaactgcattgacactgaaaaacgaaagcgtgggtagcgaaaaggattagatacccttgtagtccacgccctaaacgatgataactaagtgttgcgacgagctcgcagtgctgtagcaaacgcgttaagttatccacctgaggagtacggtcgcaagattaaaactcaaaggaatagacggggacccacacaagcagtggatcacgtggtttaattcgacaataaacggggaaccttacccagacttgacatcctaggaatactttagagatagagtagtgctcgcaagagaacctagagacaggtgctgcatggttgtcgtcagctcgtgccttgaggtgttcggttaagtccgttaacgagcgcaacccatgtccttagttacaatgtctaaggagactgccttggttaacaaggaggaaggtgtggatgacgtcaaatcagcatggcttttacgtctggggctacacacatgatacaatggcctgtacaaagagtagtgaaaccgcgaggtagaaccaatcttgaaagcaggtctcagtccggattggagtctgcaactcgactccatgaagttggaattgctagtaatcgtaaatcagatatgttacggtgaatgtgttcctgggtcttgtactcaccgcccgtcaaggcatgggaggtagtaatatcggaagtccccctagatataagggggcccatggtaggactactgactgggcttaagtcgtaacaagg

SEQ ID NO: 2 - RNA, 1418 nt, Thioreductor sp.
  source 1..1418: mol_type = rRNA
acgctagcggtgcgcctaacacatgcaagtcgagcgagagtttttgagaagcttgcttcttgaaaacaaaagcggcgaacgggtgagtaacacgttggaatctgcccctaagtcagggatagcctagtgaaaactagattaataccggatagtctctttggagtaaaaatttattgcttggggaggagcctgcgttctatcagctagttggtgaggtaagagcttaccaaggctatgacggataactggtctgagaggatgatcagtcacaatggaactgagacacggtccatactcctacgggaggcagcagtgaggaatcttccacaatggacgaaagtctgatggagcgacaccgcgtgaaggatgaaggcctaacggttgtaaacttcttttctgaaggagcataatgagagtactttaggaataagggacggctaaatatgtgccagcagccgcggtaatacatatgtctcaagcgttacccggaatcactgggtgtaaagggtttgtaggtggttttttaagtcaggtatgaaagaccggagctcaactccgagtttgtatttgaaactggagaactagaatcagggagaggtaagcgggattctaagtgtaggggtgcaatccgtagatacttagaggaacaccaaaagcgaaggcagcttactggaactgtattgacgctgagaaacgaaagcgtggggagcgaaaaggattagatacccttgtagtccacgccctaaacgatgacaactaagtgttgcgactagctcgcagtgctgtagctaacgcgttaagttgtccacctgaggagtacggtcgcaagattaaaactcaaaggaatagacggggacccacacaagcagtggatcacgtggtttaattcgataataaacggggaaccttacccagacttgacatcctaagaatgttctagagatagaatagtgctcgcaagagagcttagagacaggtgctgcatggttgtcgtcagctcgtgccttgaggtgttcggttaagtccgttaacgagcgcaacccatgtccttagttacaatgtctaaggagactgccttggttaacaaggaggaaggtgtggatgacgtcaaatcagcatggcttttacgtctggggctacacacatgatacaatggtatgtacaaagagtagtgaaatcgcgagatagaaccaatcttaaaaacatatctcagtccggattggagtctgcaactcgactccatgaagttggaattgctagtaatcgtaaatcagatatgttacggtgaatatgttcctgggtcttgtactcaccgcccgtcaaggcatgggaggtagtaatatcggaagtccccctggtaatatgggggcccatggtaggactactgactgggcttaagtcgtaacaaggtagccgta

SEQ ID NO: 3 - RNA, 1386 nt, unidentified
  source 1..1386: mol_type = rRNA
agagtttgataatggctcaagattaacgctggcggcgtgcctaacacatgcaagtcgagcggcagcgagtttttacactgaattctggaagcttctagttgaaagagaagatttattcaagaattttgtgtaaaatgtcggcgagcggcggacggctgagtaacgcgtgggaacgtaccccaaagtgagggataacgcatcgaaaggtgtgctaataccgcatatggtcttcggattaaagccttcgggcgctttgggaacggcctgcgtaagattagatagttggtggggtaatggcctaccaagtcgacgatctttaactggtttgagaggatgattcagtcagactggaactgagacacggtccagactcctacgggaggcagcagtgaggaatcttccacaatgggcgaaagcctgatggagcaacgccgcgtgcaggatgaaggccttcgggttgtaaactgcttttataagtgatgattatgacagtaacttatgaataaggattcggctaactacgtgccagcagccgcggtcatacgtaggatccgagcgttatccggagtgactgggcgtaaagagttgcgtaggtggtttaataagcgaatagtgaaatctggtggctcaaccattcagactattattcgaactgttgaactcgagagcagaagaggtagctggaatttctagtgtaggagtgaaatccgtagatattagaaggaacaccgatggcgtaggcaggctactgggctgtttctgacactgaggcacgaaagcgtggggagcgagccggattagatacccgggtagtccacgccgtaaacgatggatactagctgtttggggtatcgaccccctgagtagcgaagctaacgcgttaagtatcccgcctgtggagtacgatcgcaagattaaaacataaaggaattgacggggacccgcacaagcggtggatcatgttctttaattcgatgataaccgataaaccttaccaggtcttgacatccttggaatctttcagaaatgagagagtgctttttaagagccaagtgacaggtgatgcatggccgtcgtcagctcgtgtcgtgagatgtttggttaagtccatcaacgagcgcaacccttgtcagtagttgtatttttctactgagactgccccggtaacggggaggaaggaggggatgacgtcaggtcagtatttcccttacgtcctgggctagaaacgtgatacaatggctagtacaatgcgcagcgaagccgcgaggtgaagcaaatcgcatcaaagctagtcccagttcggattgtaggctgaaaactcgcctgcatgaagtcggaatcgctagtaatcgcggttcagcttgctgcggtgtatacgttcccggg

SEQ ID NO: 4 - RNA, 1368 nt, Helicobacter sp.
  source 1..1368: mol_type = rRNA
tttgatcctggctcaggatgaacgctagcgaaatgcctaacacatgcaagtcgaacggatcttgcgtcgtagcaatacgtagtaagattagtggcaaacgagcgagtaacgcgtgcttaacttgccccgaagatgggtataactacagagatgtagctaattcccaatatgctcacgatggtgaaattccaatgtgaggaaagatttatcgcttcgggagagtggtgcgtcctatcaggtagttggtaaggtaatggcttaccaagcctatgacgggtaaccggtctgagatgatgtccggtcgcgatgggactgagatacggcccatactcctacgggaggcagcagtggggaatcttgcacaatggacgaaagtctgatgcagcaatttcgcgtgaaggatgaagcattacggtgtgtaaacttcttttttggcagaagacgaatgacggtatgtcaagaataagagacggctaactacgtgccagcagccgcggtaatacgtaggtctcaagcgttgtccggatttactgggcgtaaagtgtccgtagtctgaattgtaagtctgttttcaaatcctacgactcaatcgtagaaagggagtggatactgcaattctggaagtatctgggggttagtggaatttccggtggagcggtgaaatgcgttgatatcggaaggaacgccgaaagcgaaagcagctaactacagaatacttgacgatgagggacgacagttcgggtagcaaacaggattagataccctggtagtccgaaccgtaaattatgcttgctagatgtttttgtcaatttattggcaggagtgtcgtaatctaacgagttaagcaagtcgcctgggtagtatattcgcaagaatgaaactcaaagggataggcgggggaacacacaagcagtggattatctagattaattggataataagccaagaatcttacctaggattgacatgtattgtgtctgcggtgaaagtcgcatatccgtagcaatacggagctttacacagatggtgcatggtcgtcgtcagctcgtgccgcaaggtgtctagttaagtctggaaacgagcgcaaccctcatgcttagttagtatgtctaagcagactgctcgggtaaccgagaggaaggagaggatgacgtcagatcctcatgcctcttacacctagggcctcatagataatacaatgggtaggtacagcgagaagcaagaccgcgaggtggagcaaatctttaaaactacccctagttcggattgtagtctggaactcgactacatgaagttggaattgctagtaatggcagatcagccatgctgccgtgaatatgtccctgttccttgcacacaccgcccgtc

SEQ ID NO: 5 - RNA, 1467 nt, Proteiniclasticum sp.
  source 1..1467: mol_type = rRNA
gagtttgatcctggctcaggatgaacgctggcggcgtgcctaacacatgcaagtcgagcggcagcgagttttacactaagttctggaagtgattcgagaattttgtgtaaaatgtcggcgagcggcggacggctgagtagcgcgtgggaacataccccaaagtgagggataactgcccgaaagggtggctaataccgcatatgatcttcggattaaaggatttatccgctttgggaatggcctgcgtcggattaggtagttggtgaggtaaaggctcaccaagccgacgatccgtaactggtttgagaggatgaccagtcagattggaactgagacacggtccagactcctacgggaggcagcagtgaggaatcttccacaatgggcgaaagcctgatggagcaacgccgcgtgcaggatgaaggccttcgggttgtaaactgcttttatgattgaggaatttgacggtagatcatgaataaggatcggctaactacgtgccagcagccgcggtcatacgtaggatccgagcgttatccggagtgactgggcgtaaagagttgcgtaggtggtttattaagtaggtgatgaaagctggtggctcaaccattcagattgttatctaaactggtaaacttgagagtagtagaggtaactggaatttctagtgtaggggtaaaatccgtagatattagaaggaacaccaatggcgtaggcaggttactggactatttctgacactgaggcacgaaagcgtggggagcgaacgggattagataccccggtagtccacgccctaaacgatggatactagctgtttgaggaatcgaccccttaagtagcgaagctaacgcgttaagtatcccgcctgtggagtacgatcgcaagattaaaacataaaggaattgacggggacccgcacaagcggtggagcatgttctttaattcgatgctaatcgatataccttaccaaggcttgacatctcgggaaggcctccgaaaggagactgtgccttttaggaacccgatgacaggtgatgcatggccgtcgtcagctcgtgtcgtgagatgtttggttaagtccattaacgagcgcaacccttgcaactagttggatttttctagttggactgccccggtaacggggaggaaggaggggatgatgtcaggtcattatttcccttacgccttgggctagaaacgtgctacaatggctggtacaaagtgcataagcgaactcgcgagagcaagcaaatcacatcaaaaccagtcccagttcggattggaggctgaaactcgcctccatgaagtcggaatcgctagtaatcgtaaatcagcaagttacggtgaatacgttcccgggtcttgtacacaccgcccgtcaaaccatgagagtgaccaacacccgaagtccgattcgtcggcctaaggcggggggcatgattggggttaagtcgtaacaaggta

SEQ ID NO: 6 - RNA, 1515 nt, unidentified
  source 1..1515: mol_type = rRNA
agagtttgatcatggctcaggacgaacgctggcggcgtgcttcatacatgcaagtcgaacgagaatctggtgcttgcaccagaggaaagtggcggacgggtgagtaatatgtaggaaatctgccctagagagggggacaacagagggaaacttctgctaataccccatatgagcgtacctgaaatggtattcttgaaaactccggtgctctaggatgagcctgcatctgattagtttgttggcggtgtaatggaccaccaagactacgatcagtagctggtttgagaggatgatcagccacaatgggactgagacacggcccatactcctacgggaggcagcagtagggaattttgcgcaatgggcgaaagcctgacgcagcaacgccgcgtgtgtgatgacgcccttcggggtgtaaaacactgtcagtagggacgaaacttgacggtacctacagaggaagcaccggctaactccgtgccagcagccgcggtaatacggagggtgcaagcgttgtccggaatcattgggcgtaaagagttcgtaggtggtttgttaagtctggtgttaaagcccgaagctcaacttcggttcggcatcggatactggcagactagaatgcggtagaggtaaagggaattcctggtgtagcggtgaaatgcgtagatatcaggaggaacatcggtggcgtaagcgctttactgggccgtaattgacactgaggaacgaaagccggggtagcaaatgggattagataccccagtagtcccggccgtaaacgatggatactaggtgttgcgggtatcgacccctgcagtgccgtagttaacgcgataagtatcccgcctggggagtacgcacgcaagtgtgaaactcaaaggaattgacggggacccgcacaagcggtggaacatgtggtttaattcgaagcaacgcgaagaaccttaccagggcttgacatctgaggaacctttgtgaaagcagagggtgctcttcggagaacctcaagacaggtggtgcacggttgtcgtcagctcgtgtcgtgagatgttgggttaagtcccgcaacgagcgcaaccctcgtcgttagttgcatatattggtatactgatatattgctctctagcgagactgccggtgataaaccggaggaaggtggggacgacgtcaaatcatcatgccccttatgtcctgggctacacacgtgttacaatggctaagacaacgagccgccaactcgcgagagtgagcaaatctcttaaacttagtctcagttcggattgcactctgcaactcgagtgcatgaagtcggaatcgctagtaaccgtagatcagcacgctgcggtgaatacgttcccgggtcttgtacacaccgcccgtcacaccatggaagtcgaccacgcccgaagcacgtgggctaaccttttggaggcagcgttctaaggcagggttggtgactggggtgaagtcgtaacaaggtagccgtaccggagggtgtggctggatcacctcctt

SEQ ID NO: 7 - RNA, 1355 nt, Nautilia profundicola
  source 1..1355: mol_type = rRNA
agagtttgatccatggctcaggatgaacgctggcggcgtgcctaacacatgcaagtcgagcggcagcgcgagtagtttactacttggcggcgagcggcggacggctgagtaacgcgtgggaatataccccaaagtgagggataactgcccgaaagggtagctaataccgcatatgatcttcggattaaaggatttatccgctttgggagtggcccgcgtcggattaggtagctggtgaggtaatggctcaccaagccgacgatccgtagctggtctgagaggatgatcagccagactgggactgagacacggcccagactcctacgggaggcagcagtgaggaatcttccacaatgggcgaaagcctgatggagcaacgccgcgtgcaggatgaaggccttcgggttgtaaactgcttttataagtgaggaatatgacggtaacttatgaataaggatcggctaactacgtgccagcagccgcggtcatacgtaggatccgagcgttatccggagtgactgggcgtaaagagttgcgtaggcggtttgttaagcgaatagtgaaacctggtggctcaaccatacagactattattcgaactggcaaactcgagagtggtagaggtcactggaatttcttgtgtaggagtgaaatccgtagatataagaaggaacaccgatggcgtaggcaggtgactagaccatttctgacgctaaggcacgaaagcgtggggagcgaaccggattagatacccgggtagtccacgccgtaaacgatggatactagctgttggaggtatcgaccccttcagtagcgaagctaacgcgttaagtatcccgcctgtggagtacggccgcaaggctaaaacataaaggaattgacggggacccgcacaagcggtggatcgtgttctttaattcgatgataaacgaagaaccctaccagggcttgacatccagggaaggtctgcgaaagcggactgtgccttttggaaccctgtgacaggtgctgcatggccgtcgtcagctcgtgtcgtgagatgtttggttaagtccatcaacgagcgcaacccttgcaactagttggatttttctagttggactgccccggtaacggggaggaaggaggggatgatgtcaggtcagtattgcccttacgtcctgggctagaaacacgatacaatggctagtacaatgcgcagcgaagccgcgaggtggagcaaatcgcatcaaagctagtcccagttcggattggaggctgaaactcgcctccatgaagtcggaatcgctagtaatcgcagatcagcaagctgcggtgaatacgttcccgggttcttgcacacaccgcccgtcaaa

SEQ ID NO: 8 - RNA, 1358 nt, unidentified
  source 1..1358: mol_type = rRNA
tttgatcatggctcaggatgaacgctggcggcgtgcctaacacatgcaagtcgagcggcagcgcgagtagtttactactttggcggcgagcggcgaacggctgagtaacgcgtcgggaatttgccccaaagtgaggaaataactgcccgaaagggtcggctaatgccgcatatgattcttcggaataaaggaattatccgcttttgggagaaacccgcgtcggattaggtagtttggtgaggtaatggctcaccaagccgacgaaccgtagctggtctgagaggatgaccagccagactggaactgagacacggtccagactcctacgggaggcagcagtgaggaatcttccacaatgggcgaaagcctgatggagcaacgccgcgtgcaggatgaaggccttcgggtttgtaaactgcttttatgattgaggaattttgacagtagattcatgaataaggatcggctaactacgtgccagcagccgcggtcatacgtaggattccgagcgttatccggagtgactgggcgtaaagagttgcgtaggcggttttgttaagtgaatagtgaaatctggtggctcaaccatacaggctattattcaaactggcaaactcgagagtggtagaggtcactggaatttcttgtgtaggagtgaaatccgtagatataagaaggaacaccgatggcgtaggcaggtgactggaccatttctgacgctaaggcacgaaagcgtggggagcgaaccggattagatacccgggtagtccacgccgtaaacgatggatactggctgttggaggtatcgaccccttcagtagcgaagctaacgcgttaagtatcccgcctgtggagtacggtcgcaagactaaaacataaaggaattgacggggacccgcacaagcggtggatcgtgttctttaattcgatgctgaacgaagaaccttaccagggcttgacatccagggaatttttgggaaaccaattagtgccttttggaaccctgtgacaggtgatgcatggccgtcgtcagctcgtgtcgtgagatgtttggttaagtccatcaacgagcgcaacccttgcaactagttggatttttctagttggactgcttcggtaacggagaggaaggaggggatgatgtcaggtcagtatttcccttacgtcctgggctagaaacacgatacaatggctagtacaatgcgcagcaaagccgcgaggtggagcaaaccgcatcaaagctagtcccagttcggattggaggctgaaactcgcctccatgaagtcggaatcgctagtaatcgcagatcagcaagctgcggtgaatacgttcccgggtcttgtacacaccgcccgtc

SEQ ID NO: 9 - RNA, 1431 nt, unidentified
  source 1..1431: mol_type = rRNA
agagtttgatcctggttcaggatgaacgctggcggcatgcctaacacatgcaagtcgatcggtaaggcccttcggggtacacgagaggcggacggctgagtaacgcgtgggaacgcaccctacactgagggataagataccgaaaggtgttctaataccgcatacggtcttcggattaaagtcttcggacggtgaaggagcggcccgcgtcatattaggtagttggtggggtaatggcctaccaagccgatgatgtgtagctggtctgagaggatgatcagccagactggaactgagaacggtccagactcctacgggaggcagcagtgaggaatattccacaatgggcgaaagcctgatggagcaatgccgcgtgcaggatgaaggccctcgggtcgtaaactgcttttattagagaagaatatgacggtaactaatgaataagggacggctaactacgtgccagcagccgcggtcatacgtaggtcccaagcgttatccggagtgactgggcgtaaagagttgcgtaggcggctaagtaagcgagtaatgaaaactatcggctcaaccggtagcctgttattcgaactgcttggctcgagattatcagaggtcgctggaattcctagtgtagcagtgaaatgcgtagatattaggaagaacaccaatggcgtaggcaggcgactggggtatttctgacgctaaggcacgaaagcgtggggagcgaaccggattagatacccgggtagtccacgccgtaaacgatggatgctaattgttcggggtatcgaccccttgagtaataaagctaacgcgttaagcatcccgcctgtggagtacggccgcaaggctaaaacataaaggaattgacggggacccgcacaagcggtggaggatgttctttaattcgatgataagcgaagaaccttaccagggcttgacatccctagaatttctccgaaaggagagagtgctttttaagaactaggtgacagatcctgcatggccgtcgtcagctcgtgtcgtgagatgtttggttaagtccatcaacgagcgcaacccttatcgttagttgtatttttctaacgagactgccccggtaacggggaggaaggaggggatgatgtcaggtcagtattggtcttacgtcctgggctagaaacgtcctacaatggctagtacaatgggcagcgaatccgcgaggtgaagcaaatcccatcaaagctagtcccagttcggattgcaggctgaaactcgcctgcatgaagtcggaatcgctagtaatcgcagatcagcacgctgcggtgaatacgttcccgggtcttgtacacaccgcccgtcaaaccatgaaagtcaggagcacccgacgtccgaatttatttcggcctaaggtgaacttggtgattggggttcagtcgtaacaaggtaacc

SEQ ID NO: 10 - RNA, 1486 nt, Bacteroides faecichinchillae
  source 1..1486: mol_type = rRNA
agagtttgatcctggctcaggatgaacgctagctacaggcttaacacatgcaagtcgaggggcagcatatttctagcaatagagatgatggcgaccggcgcacgggtgagtaacacgtatccaacctgccttatactcggggatagcctttcgaaagaaagattaatacccgatgttatagtctaaccgcatgatttgactataaaagattttcggtataagatggggatgcgttccattagattgtaggcggggtaacggcccacctagtcttcgatggataggggttctgagaggaaggtcccccacattggaactgagacacggtccaaactcctacgggaggcagcagtgaggaatattggtcaatgggcgagagcctgaaccagccaagtagcgtgaaggatgactgccctatgggttgtaaacttcttttatatgggaataaagtattccacgtgtgggattttgtatgtaccatatgaataaggatcggctaactccgtgccagcagccgcggtaatacggaggatccgagcgttatccggatttattgggtttaaagggagcgtaggtggacagttaagtcagttgtgaaagtttgcggctcaaccgtaaaattgcagttgatactggctgtcttgagtacagtagaggtgggcggaattcgtggtgtagcggtgaaatgcttagatatcacgaagaactccgattgcgaaggcagctcactggactgcaactgacactgatgctcgaaagtgtgggtatcaaacaggattagataccctggtagtccacacagtaaacgatgaatactcgctgtttgcgatatacagtaagcggccaagcgaaagcattaagtattccacctggggagtacgccggcaacggtgaaactcaaaggaattgacgggggcccgcacaagcggaggaacatgtggtttaattcgatgatacgcgaggaaccttacccgggcttaaattgcaaatgaataatctggaaacaggttagccgcaaggcatttgtgaaggtgctgcatggttgtcgtcagctcgtgccgtgaggtgtcggcttaagtgccataacgagcgcaacccttatctttagttactaacaggtcatgctgaggactctagagagactgccgtcgtaagatgtgaggaaggtggggatgacgtcaaatcagcacggcccttacgtccggggctacacacgtgttacaatggggggtacagaaggccgctacctggtgacaggatgctaatccctaaaacctctctcagttcggatcgaagtctgcaacccgacttcgtgaagctggattcgctagtaatcgcgcatcagccatggcgcggtgaatacgttcccgggccttgtacacaccgcccgtcaagccatgaaagccgggggtacctgaagtacgtaaccgcaaggagcgtcctagggtaaaactggtaattggggctaagtcgtaacaaggtaacc

SEQ ID NO: 11 - RNA, 1384 nt, Streptococcus vestibularis
  source 1..1384: mol_type = rRNA
gcggcgagcctaatacacgcaagtagaaacgctgaagggagagagcttcgctcttcttcggacgagctcgcgaaacgggcgagtaacgcgtaggtaacccgcctccgtagcgggggataactattcggaaacgatagctaataccgcataacaataggtgaacacatgtcatttatttgaaaggggcaatcgctccactacaagatggacctgcgttgtattagctagtaggtgaggtaacggctcacctaggcgacgatacatagccgacctgagagggtgatcggccacactgggactgagacacggcccagactcctacgggaggcagcagtagggaatcttcggcaatgggggcaaccctgaccgagcaacgccgcgtgagtgaagaaggttttcggaacgtaaagctctgttgtaagtcaagaacgagtgtgagagtggaaagttcacactgtgacggtagcttaccagaaagggacggctaactacgtgccagcagccgcggtaatacgtaggtcccgagcgttgtccggatttattgggcgtaaagcgagcgcaggcggtttgataagtctgaagttaaaggctgtggctcaaccatagttcgctttggaaactgtcaaacttgagtgcagaaggggagagtggaattccatgtgtagcggtgaaatgcgtagatatatggaggaacaccggtggcgaaagcggctctctggtctgtaactgacgctgaggctcgaaagcgtggggagcgaacaggattagataccctggtagtccacgccgtaaacgatgagtgctaggtgttggatcctttccgggattcagtgccgcagctaacgcattaagcactccgcctggggagtacgaccgcaaggttgaaactcaaaggaattgacgggggcccgcacaagcggtggagcatgtggtttaattcgaagcaacgcgaagaaccttaccaggtcttgacatcccgatgctatttctagagatagaaagttacttcggtacatcggtgacaggtggtgcatggttgtcgtcagctcgtgtcgtgagatgttgggttaagtcccgcaacgagcgcaacccctattgttagttgccatcattcagttgggcactctagcgagactgccggtaataaaccggaggaaggtggggatgacgtcaaatcatcatgccccttatgacctgggctacacacgtgctacaatggttggtacaacgagttgcgagtcggtgacggcaagctaatctcttaaagccgaatctcagttcggattgtaggctgcgaactcgcctacgtaaagtcggaaatcgctaggaatcgcgaatcagcacgccgcggtaaagacgttcccgggccttgcccccaccgccc

SEQ ID NO: 12 - RNA, 1434 nt, Parasutterella excrementihominis
  source 1..1434: mol_type = rRNA
cgctggcggaacgctttacacatgcaagtcgaacctttacggggggaggagcttgctccagcccaacaacgagtggcgaacgggtgaggaatacatcggagcgtgaccgctcgtgggggacaaccagccgaaaggttggctaataccgcatgagttctacggaagaaagagggggacccgcaagggcctctcgcgagcggagcggccgatgactgattagcctgttggtgaggtaacggctcaccaaagcaacgatcagtagctggtctgagaggacgaccagccacactgggactgagacacggaccagactcctacgggaggcagcagtggggaattttggacaatgggcgcaagcctgatccagctattccgcgtgtgggatgaaggccctcgggttgtaaaccacttttgtagagaacgaaaagacatcttcgaataaaggatgttgctgacggtactctaagaataagcaccggctaactacgtgccagcagccgcggtaatacgtagggtgcgagcgttaatcggaattactgggcgtaaagggtgcgcaggcggttgagtaagacagatgtgaaatccccgagcttaactcgggaatggcatatgtgactgctcgactagagtgtgtcagagggaggtggaattccacgtgtagcagtgaaatgcgtagatatgtggaagaacaccgatggcgaaggcagcctcctgggacataactgacgctctggcacgaaagcgtggggagcaaacaggattagatactctggtagtccacgccctaaacgatgttaactagttgttgggatgtaataatctcagtaacgcagccaacgcgagaagttaaccgcctgggaagtacggtcgcaagactaaaactcaaaggaattgacggggacccgcacaagcggtggatgatgtggattaattcgatgcaacgcgaaaaaccttacctacccttgacatgtcaggaagctcttgtaatgagagcgtgtccgcaagggagcctgaacacaggtggtgcatggctgtcgtcagctcgtgtcgtgagatgttgggttaagtcccgcaacgagcgcaatccttgtcactagttgcttcgaaagggcactctagtgagactgccggtgacaaaccggaggaaggtggggatgacgtcaagtcctcatggcccttatgggtagggcttcccacgtcatacaatggtcggaacagagggcagggaagccgtgaggcggagccaatcccagaaaaccgatcgtagtccggattgcagtttgcaacttgactgcatgaagttggaatcgctagtaatcgcggatcagcatgccgcggtgaatacgttcccgggtcttgtacaccccgcccgtcaaccaatgggagtggtgtttcccagaagtcgttagcctaaccgcaaggagggcggcgacc

SEQ ID NO: 13 - RNA, 1440 nt, Eubacterium eligens
  source 1..1440: mol_type = rRNA
ggcgtgcttaacacatgcaagtcgagcgaagcacttaggaaagattcttcggatgatttcctatttgactgagcggcggacgggtgagtaacgcgtgggtaacctgcctcatacagggggataacagttagaaatgactgctaataccgcataagaccacagcactgcatggtgcaggggtaaaaactccggtggtatgagatggacccgcgtctgattagttagttggtggggtaacggcctaccaaggcgacgatcagtagccgacctgagagggtgaccggccacattgggactgagacacggcccaaactcctacgggaggcagcagtggggaatattgcacaatgggggaaaccctgatgcagcgacgccgcgtgagcgaagaagtatttcggtatgtaaagctctatcagcagggaagaaaatgacggtacctgactaagaagccccggctaaatacgtgccagcagccgcggtaatacgtatggagcaagcgttatccggatttactgggtgtaaagggagtgtaggtggccatgcaagtcagaagtgaaaatccggggctcaaccccggaactgcttttgaaactgtaaggctagagtgcaggaggggtgagtggaattcctagtgtagcggtgaaatgcgtagatattaggaggaacaccagtggcgaaggcggctcactggactgtaactgacactgaggctcgaaagcgtggggagcaaacaggattagataccctggtagtccacgccgtaaacgatgaatactaggtgtcggggcccataagggcttcggtgccgcagcaaacgcaataagtattccacctggggagtacgttcgcaagaatgaaactcaaaggaattgacggggacccgcacaagcggtggagcatgtggtttaattcgaagcaacgcgaagaaccttaccaagtcttgacatcccactgaccggacagtaatgtgtcctttccttcgggacagtggtgacaggtggtgcatggttgtcgtcagctcgtgtcgtgagatgttgggttaagtcccgcaacgagcgcaacccctatccttagtagccagcagtaagatgggcactctagggagactgccagggataacctggaggaaggtggggatgacgtcaaatcatcatgccccttatgacttgggctacacacgtgctacaatggcgtaaacaaagtgaagcgaagtcgtgaggccaagcaaatcacaaaaataacgtctcagttcggattgtagtctgcaactcgactacatgaagctggaatcgctagtaatcgcagatcagaatgctgcggtgaatacgttcccgggtcttgtacacaccgcccgtcacaccatgggagtcgaaaatgcccgaagtcggtgacctaacgaaagaaggagccgccgaaggcaggtttgataactggggtgaa

SEQ ID NO: 14 - RNA, 1380 nt, unidentified
  source 1..1380: mol_type = rRNA
gacgaactctggcggcgcgcctaacacatgcaagtcgaacggagcttagagagcttgctttttaagcttagtggcgaacgggtgagtaacgcgtggataatctacccttaagatggggataacggctggaaacggtcgctaataccgaatacgctcccgattttatcggtggggggaaagatggcctctgcttgcaagctatcgcttaaggatgagtccgcgtcccattagctagttggcggggtaacggcccaccaaggcgacgatgggtagccggtctgagaggatgaccggccacactggaactggaacacggtccagactcctacgggaggcagcagtggggaatattgcgcaatgggcgaaagcctgacgcagcgacgccgcgtgagggatgaaggttctcggatcgtaaacctctgtcaggggggaagaaaccccctcgtgtgaataatgcgagggcttgacggtacccccaaaggaagcaccggctaactccgtgccagcagccgcggtaatacggagggtgcaagcgttaatcggaatcactgggcgtaaagcgcacgtaggcggcttggtaagtcaggggtgaaatcccacagcccaactgtggaactgcctttgatactgccaggcttgagtaccggagagggtggcggaattccaggtgtaggagtgaaatccgtagatatctggaggaacaccggtggcgaaggcggccacctggacggtaactgacgctgaggtgcgaaagcgtgggtagcaaacaggattagataccctggtagtccacgctgtaaacgatgggtgctgggtgctgggatgtatgtctcggtgccgtagctaacgcgataagcaccccgcctggggagtacggtcgcaaggctgaaactcaaagaaattgacgggggcccgcacaagcggtggagtatgtggtttaattcgatgcaacgcgaagaaccttacccaggcttgacatctagggaacccttcggaaatgaaggggtgcccttcggggagccctaagacaggtgctgcatggctgtcgtcagctcgtgccgtgaggtgttgggttaagtcccgcaacgagcgcaacccctatcttcagttgccagcaggtaaggctgggcactctggagagaccgccccggtcaacggggaggaaggtggggacgacgtcaagtcatcatggcccttacgcctggggctacacacgtactacaatggcgcgcacaaagggtagcgagaccgcgaggtggagccaatcccaaaaaacgcgtcccagtccggattggagtctgcaactcgactccatgaagtcggaatcgctagtaattcgagatcagcatgctcgggtgaatgcgttcccgggccttgcac

SEQ ID NO: 15 - RNA, 1347 nt, Roseburia faecis
  source 1..1347: mol_type = rRNA
gagtggcggacgggtgagtaacgcgtgggtaacctgcctcatacagggggataacagttagaaatgactgctaataccgcataagcgcacagtaccgcatggtacggtgtgaaaaactccggtggtatgagatggacccgcgtctgattagctagttggcggggtaacggcccaccaaggcgacgatcagtagccgacctgagagggtgaccggccacattgggactgagacacggcccaaactcctacgggaggcagcagtggggaatattgcacaatgggcgaaagcctgatgcagcgacgccgcgtgaacgaagaagtatttcggtatgtaaagttctatcagcagggaagataatgacggtacctgactaagaagcaccggctaaatacgtgccagcagccgcggtaatacgtatggtgcaagcgttatccggatttactgggtgtaaagggagcgcaggcggtacggcaagtctgatgtgaaagcccggggctcaaccccggtactgcattggaaactgtcgaactagagtgtcggaggggtaagcggaattcctagtgtagcggtgaaatgcgtagatattaggaggaacaccagtggcgaaggcggcttactggacgataactgacgctgaggctcgaaagcgtggggagcaaacaggattagataccctggtagtccacgccgtaaacgatgaatactaggtgtcgggtcccacagggattcggtgccgcagcaaacgcaataagtattccacctggggagtacgttcgcaagaatgaaactcaaaggaattgacggggacccgcacaagcggtggagcatgtggtttaattcgaagcaacgcgaagaaccttaccaagtcttgacatcccgatgaccggtacttaaccgtaccttttcttcggaacatcggtgacaggtggtgcatggttgtcgtcagctcgtgtcgtgagatgttgggttaagtcccgcaacgagcgcaacccctgttcttagtagccagcggtttggccgggcactctaggaagactgccagggataacctggaggaaggcggggatgacgtcaaatcatcatgccccttatgacttgggctacacacgtgctacaatggcgtaaacaaagggaagcaaagctgtgaggccgagcaaatctcaaaaataacgtctcagttcggattgtagtctgcaactcgactacatgaagctggaatcgctagtaatcgcgaatcagaatgtcgcggtgaatacgttcccgggtcttgtacacaccgcccgtcacaccatgggagttggaaatgcccgaagtcagtgacccaaccgcaaggagggagctgccga

SEQ ID NO: 16 - RNA, 1449 nt, Blautia sp.
  source 1..1449: mol_type = rRNA
atgaacgctggcggcgtgcctaacacatgcaagtcgagcgaagcacttgcaaatgatccttcgggtgattttgctggtgactgagcggcggacgggtgagtaacgcgtgggtaacctgcctcatacagggggataacagttagaaatgactgctaataccgcataagcgcacagtaccacatggtacggtgtgaaaaactccggtggtatgagatggacccgcgtctgattagctagttggcggggtaacggcccaccaaggcgacgatcagtagccgacctgagagggtgatcggccacattgggactgagacacggcccaaactcctacgggaggcagcagtggggaatattgcacaatgggggaaaccctgatgcagcaacgccgcgtgagtgaagaagtatttcggtatgtaaagctctatcagcagggaagataatgacggtacctgactaagaagccccggctaactacgtgccagcagccgcggtaatacgtagggggcaagcgttatccggatttactgggtgtaaagggagcgtagacggcgcagcaagtctgatgtgaaaggcaggggcttaacccctggactgcattggaaactgctgtgcttgagtgccggaggggtaagcggaattcctagtgtagcggtgaaatgcgtagatattaggaggaacaccagtggcgaaggcggcttactggacggtaactgacgttgaggctcgaaagcgtgggggagcaaacaggatttagataccctggtagtccacgccgtaaacgatgaatactaggtgtcagggagcacagctccttttggtgccgccgcaaaggcattaagtattccaccgggggagtacgttcgcaagaatgaaactcaaaggaattgacggggacccgcacaagcggtggagcatgtggtttaattcgaagcaacgcgaagaaccttaccaaatcttgacatccctctgaccgggacttaaccgtccctttctttcgggacaggggagacaggtggtgcatggttgtcgtcagctcgtgtcgtgagatgttgggttaagtcccgcaacgagcgcaacccctatccttagtagccagcacgcagtggtgggcactctgaggagactgccagggataacctggaggaaggcggggatgacgtcaaatcatcatgccccttatgatttgggctacacacgtgctacaatggcgtaaacaaagggaagcgaacccgcgagggtgggcaaatctcaaaaataacgtcccagttcggactgcagtctgcaactcgactgcaggaagctggaatcgctagtaatcgcggatcagaatgccgcggtgaatacgttcccgggtcttgtacacaccgcccgtcacaccatgggagtcagtaacgcccgaagtcagtgacctaaccgcaagggaggagctgccgaaggcgggaccgatga

SEQ ID NO: 17 - RNA, 1427 nt, Phocaeicola sp.
  source 1..1427: mol_type = rRNA
ctcaggatgaacgctagctacaggcttaacacatgcaagtcgaggggcagcatggtcttagcttgctaaggctgatggcgaccggcgcacgggtgagtaacacgtatccaacctgccgtctactcttggccagccttctgaaaggaagattaatccaggatgggatcatgagttcacatgtccgcatgattaaaggtattttccggtagacgatggggatgcgttccattagatagtaggcggggtaacggcccacctagtcaacgatggataggggttctgagaggaaggtcccccacattggaactgagacacggtccaaactcctacgggaggcagcagtgaggaatattggtcaatgggcgatggcctgaaccagccaagtagcgtgaaggatgactgccctatgggttgtaaacttcttttataaaggaataaagtcgggtatgcatacccgtttgcatgtactttatgaataaggatcggctaactccgtgccagcagccgcggtaatacggaggatccgagcgttatccggatttattgggtttaaagggagcgtagatggatgtttaagtcagttgtgaaagtttgcggctcaaccgtaaaattgcagttgatactggatgtcttgagtgcagttgaggcaggcggaattcgtggtgtagcggtgaaatgcttagatatcacgaagaactccgattgcgaaggcagcctgctaagctgcaactgacattgaggctcgaaagtgtgggtatcaaacaggattagataccctggtagtccacacggtaaacgatgaatactcgctgtttgcgatatactgcaagcggccaagcgaaagcgttaagtattccacctggggagtacgccggcaacggtgaaactcaaaggaattgacgggggcccgcacaagcggaggaacatgtggtttaattcgatgatacgcgaggaaccttacccgggcttaaattgcagatgaattacggtgaaagctgtaagccgcaaggcatctgtgaaggtgctgcatggttgtcgtcagctcgtgccgtgaggtgtcggcttaagtgccataacgagcgcaacccttgttgtcagttactaacaggttttgctgaggattctgacaagactgccatcgtaagatgtgaggaaggtggggatgacgtcaaatcagcacggcccttatgtccggggctacacacgtgttacaatggggggtacagagggctgctaccacgcaagtggatgccaatcccaaaaacctctgtcagttcggattgaagtctgcaacccgacttcatgaagctggattcgctagtaatcgcgcatcagccacggcgcggtgaatacgttcccgggccttgtacactccgcccgtcaatccatgggagccgggggtacctgaagtgcgtaaccgcaaggag

SEQ ID NO: 18 - RNA, 1453 nt, unidentified
  source 1..1453: mol_type = rRNA
ggatgaacgctggcggcgtgcttaacacatgcaagtcgaacgaagcaatctagcggaagttttcggatggaagctggattgactgagtggcggacgggtgagtaacgcgtgggtaacctgcctcacactgggggacaacagttagaaatgactgctaataccgcataagcgcacaggaccgcatggtccggtgtgaaaaactccggtggtgtgagatggacccgcgtttgattagctagttggtggggtaacggcctaccaaggcgacgatcaatagccgacctgagagggtgaccggccacattgggactgagacacggcccaaactcctacgggaggcagcagtggggaatattgcacaatgggggaaaccctgatgcagcgacgccgcgtgagtgaagaagtatttcggtatgtaaagctctatcagcagggaagaaaatgacggtacctgactaagaagccccggctaactacgtgccagcagccgcggtaatacgtagggggcaagcgttatccggatttactgggtgtaaagggagcgtagacggtaaagcaagtctgaagtgaaagcccggggctcaaccccgggactgctttggaaactgtttaactagagtgctggagaggtaagcggaattcctagtgtagcggtgaaaatgcgtagatattacgaggaacacccattggcgaagggggcttattggacaagtaactgacgttgaggcttgaaaagcgtggggagcaaacaggattagataccctggtagtccaccccgtaaacgatgaatattaggtgtgtggggacaaagtcgttcggtgccgtcgcaaacgcaataagtattccacgtggggagtacgttcgcaagaaagaaactcaaaggaattgacgcggacccgcacaagcggtggagcacgtggtttaatttgaagcaacgcgaagaaccttaccaaatcttgacatccctctgaccggcgagtaatgtctcctttctttcgggacagaggagacaggtggtgcatggttgtcgtcagctcgtgtcgtgagatgttgggttaagtcccgcaacgagcgcaacccttatcttaagtagccagcagttcggctgggcactcttgggagactgccagggataacctggaggaaggtggggatgacgtcaaatcatcatgccccttatgatttgggctacacacgtgctacaatggcgtaaacaaagagaggcgagaccgcgaggtggagcaaatctcaaaaataacgtctcagttcggactgcaggctgcaactcgcctgcacgaagctggaatcgctagtaatcgcgaatcagaatgtcgcggtgaatacgttcccgggtcttgtacacaccgcccgtcacaccatgggagtcagtaatgcccgaagtcagtgacccaaccgaaaagagggagctgccgaaggcaggaccgataactg

SEQ ID NO: 19 - RNA, 1418 nt, Peptoniphilus sp.
  source 1..1418: mol_type = rRNA
aacacatgcaagtcgagcgatgaaattttccctgaacccttcggggtgaagacaaaatggattagcggcggacgggtgagtaacacgtgagtaacctgccttagacattgtgatagcctcgggaaaccgggattaataccgaataaaatcataggtgcacatgcactaatgatcaaaactccggtggtctaagatggactcgcgtcccattagctagttggtagggtaacggcctaccaaggcgacgatgggtagccggcctgagagggtgaacggccacattggaactgagaaacggtccaaactcctacgggaggcagcagtggggaatattgcacaatggagggaactctgatgcagcgacgccgcgtgaacgaagaaggctttcgagtcgtaaagttcttttatatgggaagataatgacggtaccataagaaaaagctccggctaactacgtgccagcagccgcggtaatacgtagggggctagcgttgtccggaatcactgggcgtaaagggttcgcaggcggaaatgcaagtcaggtgtaaaaggcagtagcttaactactgtaagcatttgaaactgcatatcttgagaagagtagaggtaagtggaatttttagtgtagcggtgaaatgcgtagatattaaaaagaataccggtggcgaaggcgacttactgggctcattctgacgctgaggaacgaaagcgtgggtagcaaacaggattagataccctggtagtccacgctgtaaacgatgagtgctaggtgtcggcgtaagtcggtgccgcagttaacacaataagcactccgcctggggagtacgtgcgcaagcatgaaactcaaaggaattgacggggacccgcacaagcagcggagcatgtggtttaattcgaagcaacgcgaagaaccttaccagggcttgacatactgaggacgtatttagagataaatattcctcttcggaggcctcaatacaggtggtgcatggttgtcgtcagctcgtgtcgtgagatgttgggttaagtcccgcaacgagcgcaacccttatctttagttgccagcatttcggatgggaactctaaagagactgccgatgacaaatcggaggaaggtggggatgacgtcaaatcatcatgccctatatgccctgggttacacacgtgctacaatggaaggtacaaagggaagcaagatagtgatattaagcaaacctcaaaaagcctttcccagttcggattgtactctgcaactcgagtacatgaagatggagttgctagtaatcgcagatcagaatgctgtggtgaatgcgttcccgggtcttgtacacaccgcccgtcacaccatgggagccgggggtacctgaagtgcgtaaccgcgaggagcgccctagggtaaaactggtgactggggctaa

SEQ ID NO: 20 - RNA, 1413 nt, Faecalibacterium prausnitzii
  source 1..1413: mol_type = rRNA
gctggcggcgcgcctaacacatgcaagtcgcccttgcgagagagagcttgctttctcgagcgagtggcgaacgggtgagtaacgcgtgaggaacctgcctcaaagagggggacaacagttggaaacgactgctaataccgcataagcccacgacccggcatcgggtagagggaaaaggagcaatccgctttgagatggcctcgcgtccgattagctagttggtgaggtaacggcccaccaaggcgacgatcggtagccggactgagaggttgaacggccacattgggactgagacacggcccagactcctacgggaggcagcagtggggaatattgcacaatgggggaaaccctgatgcagcgacgccgcgtggaggaagaaggtcttcggattgtaaactcctgttgttgaggaagataatgacggtactcaacaaggaagtgacggctaactacgtgccagcagccgcggtaaaacgtaggtcacaagcgttgtccggaattactgggtgtaaagggagcgcaggcgggaagacaagttggaagtgaaatccatgggctcaacccatgaactgctttcaaaactgtttttcttgagtagtgcagaggtaggcggaattcccggtgtagcggtggaatgcgtagatatcgggaggaacaccagtggcgaaggcggcctactgggcaccaactgacgctgaggctcgaaagtgtgggtagcaaacaggattagataccctggtagtccacactgtaaacgatgattactaggtgttggaggattgacccttccagcgccgcagtaatcacaataagtaatccacatggcgagtacgaccgcaaggttgagactcaaaggaattgacgggggcccgcacaagcagtggagtatgtggtgtaattcgacgcaacgcgaagaaccttagcaagtcttgacatcctgcgacggttctggaaacagaactttccttcgggacgcagagacaggtggtgcatggttgtcgtcagctcgtgtcgtgagatgttgggttaagtcccgcaacgagcgcaacccttatggtcagttactacgcaagaggactctggccagactgccgtagacaaaacggaggaaggtggggatgacgtcaaatcatcatgccctttatgacttgggttacacacgtactacaatggcgttaaacaaagagaagcaagaccgcgaggtggagcaaaactcagaaacatcgtctcagtttggaatgcaggctgcaactcgcctgcacgaagtcggaattgctagtaatcgcggatcagcatggtgcggtgaatacgttcccgggccttgtacacaccgcccgtcacaccatgagagccggggggacccgaagtcggtagtctaactgtaaggaggacgccgccgaaggtaaaact

SEQ ID NO: 21 - RNA, 1457 nt, unidentified
  source 1..1457: mol_type = rRNA
gacgaacgctgtcggcgcgcttaacacatgcaagtcgagcgatgaaattttgacagatcccttcggggtgaagataaaatggattagcggcggacgggtgagtaacgcgtgggtaacctgccccatacagggggataacagttagaaatgactgctaataccgcataagaccacagcgccgcatggtgcaggggtaaaaactccggtggtatgggatggacccgcgtctgattagctagttggcggggtaacggcccaccaaggcgacgatcagtagccgacctgagagggtgaccggccacattgggactgagacacggcccaaactcctacgggaggcagcagtggggaatattgcacaatgggggaaaccctgatgcagcgacgccgcgtgagtgatgaagtatttcggtatgtaaagctctatcagcagggaagaaaatgacggtacctgactaagaagccccggctaactacgtgccagcagccgcggtaatacgtagggggcaagcgttatccggatttactgggtgtaaagggagcgtagacggctgtgcaagtctggagtgaaagcccggggctcaaccccgggactgctttggaaactgtacggctggagtgctggagaggcaagcggaattcctagtgtagcggtgaaatgcgtagatattaggaggaacaccagtggcgaaggcggcttgctggacagtaactgacgttgaggctcgaaagcgtggggagcaaacaggattagataccctggtagtccacgccgtaaacgatgaatgctaggtgtcggggagcaaagctcttcggtgccgccgcaaacgcaataagcattccacctggggagtacgttcgcaagaatgaaactcaaaggaattgacggggacccgcacaagcggtggagcatgtggtttaattcgaagcaacgcgaagaaccttaccaagtcttgacatccccctgaccggcaagtaatgttgcctttccttcgggacaggggagacaggtggtgcatggttgtcgtcagctcgtgtcgtgagatgttgggttaagtcccgcaacgagcgcgacccttatcctcagtagccagcaggtgaagctgggcactctgtggagactgccagggataacctggaggaaggtggggacgacgtcaaatcatcatgccccttatgacttgggctacacacgtgctacaatggcgtaaacaaagggaagcgagagggtgacctggagcaaatcccaaaaataacgtctcagttcggattgtagtctgcaactcgactacatgaagctggaatcgctagtaatcgcgaatcagcatgtcgcggtgaatacgttcccgggtcttgtacacaccgcccgtcacaccatgggagtcagcaacgcccgaagccggtgacctaaccgcaaggaaggagccgtcgaaggcggggcaggtaactggggtgaa

SEQ ID NO: 22 - RNA, 1426 nt, Bacteroides thetaiotaomicron
  source 1..1426: mol_type = rRNA
gcttaacacatgcaagtcggggggcagcattcctttttgcttgcaaactggagatggcgaccggcgcacgggtgagtaacacgtatccaacctgccgataactcggggatagcctttcgaaagaaagattaatacccgatggtataatcagaccgcatggtcttgttattaaagaatttcggttatcgatggggatgcgttccattaggcagttggtgaggtaacggctcaccaaaccttcgatggataggggttctgagaggaaggtcccccacattggaactgagacacggtccaaactcctacgggaggcagcagtgaggaatattggtcaatgggcgcaggcctgaaccagccaagtagcgtgaaggatgactgccctatgggttgtaaacttcttttatatgggaataaagttttccacgtgtggaattttgtatgtaccatatgaataaggatcggctaactccgtgccagcagccgcggtaatacggaggatccgagcgttatccggatttattgggtttaaagggagcgtacgtggacagttaagtcagttgtgaaagtttgcggctcaaccgtaaaattgcagttgatactggctgtcttgagtacagtagaggtgggcggaattcgtggtgtagcggtgaaatgcttagatatcacgaagaactccgattgcgaaggcagctcactggactgcaactgacactgatgctcgaaagtgtgggtatcaaacaggattagataccctggtagtccacacagtaaacgatgaatactcgctgtttgcgatatacagtaagcggccaagcgaaagcattaagtattccacctggggagtacgccggcaacggtgaaactcaaaggaattgacgggggcgcgcacaagcggaggaacatgtggtttaattagatgatacgcgaggaaccttacccgggcttaaattgcatttgaatatattggtaacagtatagtcgtaagacaaatgtgaaggtgctgcatggttgtcgtcagctcgtgccgtgaggtgtcggcttaagtgccataacgagcgcaacccttatctttagttattaacaggtcatgctgaggactctagagagactgccgtggtaagatgtgaggaaggtggggatgacgtcaaatcagcacggcccttacgtccggggctacacacgtgttacaatggggggtacagaaggcaggtacctggtgacaggatggtaatcccaaaagcctttgtcagttaggatggaagtctgcaacccgaattcgtgaagctggattagctagtaatcgcgcatcagccagggtgcggtgaatacgttcccgggccttgtacaccccgcccgtcaagccatgaaagccgggggtacgtgaagtacgtaaaaacaaggagcgtcctagggtaaaactggtaat

SEQ ID NO: 23 - RNA, 1523 nt, unidentified
  source 1..1523: mol_type = rRNA
agagtttgatcctggctcaggatgaacgctggcggcgtgcctaacacatgcaagtcgaacggagtcgttttggaaaatccttcgggattggaattctcgacttagtggcggacgggtgagtaacgcgtgagcaatctgcctttaagagggggataacagtcggaaacggctgctaataccgcataaagcattaaattcgcatgtttttgatgccaaaggagcaatccgcttctagatgagctcgcgtctgattagctggttggcggggtaacggcccaccaaggcgacgatcagtagccggactgagaggttgaacggccacattgggactgagacacggcccagactcctacgggaggcagcagtggggaatattgcgcaatgggggaagccctgacgcagcaacgccgcgtgattgaagaaggccttcgggttgtaaagatctttaatcagggacgaaacaaatgacggtacctgaagaataagctccggctaactacgtgccagcagccgcggtaatacgtagggagcaagcgttatccggatttactgggtgtaaagggcgcgcaggcgggccggcaagttggaagtgaaatctatgggcttaacccataaactgctttcaaaactgctggtcttgagtgatggagaggcaggcggaattccgtgtgtagcggtgaaatgcgtagatatacggaggaacaccagtggcgaaggcggcttgctggacattaactgacgctgaggcgcgaaagcgtggggagcaaacaggattagataccctggtagtccacgccgtaaacgatggatactaggtgtgggaggtattgaccccttccgtgccgcagttaacacaataagtatcccacctggggagtacggccgcaaggttgaaactcaaaggaattgacgggggcccgcgcaagcagtggagtatgtggtttaattcgaagcaacgcgaagaaccttaccaggtcttgacatcccgatgaccgccttagagataaggcttttcttcggaacatcggtgacaggtggtgcatggttgtcgtcagctcgtgtcgtgagatgttgggttaagtcccgcaacgagcgcaacccttacggttagttgatacgcaagatcactctagccggactgccgttgacaaaacggaggaaggtggggacgacgtcaaatcatcatgccccttatgacctgggctacacacgtactacaatggcagtcatacagagggaagcaaaaccgcgaggtggagcaaatccctaaaagctgtcccagttcagattgcaggctgcaacccgcctgcatgaagtcggaattgctagtaatcgcggatcagcatgccgcggtgaatacgttcccgggccttgtacacaccgcccgtcacaccatgagagccgtcaatacccgaagtccgtagcctaaccgtaaggagggcgcggccgaaggtaggggtggtaattagggtgaagtcgtaacaaggtagccgtatcggaaggtgcggctggatcacctcctt

SEQ ID NO: 24 - RNA, 1456 nt, Dialister propionicifaciens
  source 1..1456: mol_type = rRNA
cttacacatgcagtcgaacgggaagagatgaagagcttgctctttatcgaatccagtggcaaacgggtgagtaacacgtaaacgacctgccttcaggatggggacaacagacggaaacgactgctaataccgaatacgttccacgggccgcatgacctgtggaagaaagggtagcctctacctgtaagctatcgcctgaagaggggtttgcgtctgattaggcagttggtggggtaacggcccaccaaaccaacgatcagtagccggtctgagaggatgaacggccacactggaactgagacacggtccagactcctacgggaggcagcagtggggaatcttccgcaatggacgaaagtctgacggagcaacgccgcgtgagtgaagacggccttcgggttgtaaagctctgtgatccgggacgaaagagcctgaggtgaatagcctaaggaagtgacggtaccggaaaagcaagccacggctaactacgtgccagcagccgcggtaatacgtaggtggcaagcgttgtccggaattattgggcgtaaagcgcgcgcaggcggcttcctaagtccatcttaaaagtgcggggcttaaccccgtgatgggatggaaactgggaagctggagtatcggagaggaaaggtggaattcctagtgtagcggtgaaatgcgtagagattaggaagaacaccggtggcgaaggcgactttctggacgaaaactgacgctgaggcgcgaaagcgtggggagcaaacaggattagataccctggtagtccacgccgtaaacgatggataggggggggggtgggggctccccccttctgtgccggagttaacgcaataagtatcccgcctgggaagtacgatcgcaagattaaaactcaaaggaattgacgggggcccgcacaagcggtggagtatgtggtttaattcgacgcaacgcgaagaaccttaccaggtcttgacattgatcgcaattttcagaaatgagaagttctccttcgggagacgagaaaacaggtggtgcacggctgtcgtcagctcgtgtcgtgagatgttgggttaagtcccgcaacgagcgcaacccctatcatttgttgccagcacgtaaaggtggggactcaaatgagaccgccgcagacaatgcggaggaaaggtggggatgacgtcaagtcatcatgccccttatgacctgggctacacacgtactacaatgggtgtcaacaaagagaagcgaaagggcgacctggagccaacctcaaaaacacacccccagttcagatcgcaggctgcaactcgcctgcgtgaagcaggaatcgctagtaatcgcgggtcagcataccgcggtgaatacgttcccgggccttgtacacaccgcccgtcacactatgagagtcagaaacacccgaagccggtgaggtaaccgcaaggagccagccgtcgaaggcgag